European Patent Application EP 4 442 705 A1, published October 9, 2024. Title: Dosage. Applicant: CITRYLL B.V. The sequence listing filed with the application follows.

SEQUENCE LISTING (56 sequences)

SEQ ID NO: 1 - protein, 8 aa, synthetic construct
  REGION 1..8: note = CDR1 of msVH22.101 and hVH22.101(HC)x
GYTFTNYG

SEQ ID NO: 2 - protein, 8 aa, synthetic construct
  REGION 1..8: note = CDR2 of msVH22.101 and hVH22.101(HC)x
INTYSGEA

SEQ ID NO: 3 - protein, 15 aa, synthetic construct
  REGION 1..15: note = CDR3 of msVH22.101 and hVH22.101(HC)x
LRGYTYQSFDEGGDY

SEQ ID NO: 4 - skipped

SEQ ID NO: 5 - protein, 9 aa, synthetic construct
  REGION 1..9: note = CDR3 of msVL22.101 and hVL22.101(LC)y
WQGTHFPYT

SEQ ID NO: 6 - protein, 11 aa, Homo sapiens
QSLLDTDGKTY

SEQ ID NO: 7 - protein, 11 aa, Homo sapiens
QSLLDSDAKTY

SEQ ID NO: 8 - protein, 11 aa, Homo sapiens
QSLLDTDAKTY

SEQ ID NO: 9 - protein, 11 aa, Homo sapiens
QSLLDADGKTY

SEQ ID NO: 10 - protein, 11 aa, Homo sapiens
QSLLDNDGKTY

SEQ ID NO: 11 - protein, 122 aa, synthetic construct
  REGION 1..122: note = hVH22.101f
RIQLVQSGAEVKKPGASVKVSCKASGYTFTNYGMHWVRQAPGQGLEWMGWINTYSGEATYAQKFQGRVTMTRDTSISTAYMELSRLRSDDTAVYYCLRGYTYQSFDEGGDYWGQGTLVTVSS

SEQ ID NO: 12 - protein, 122 aa, Homo sapiens
RIQLVQSGAEVKKPGASVKVSCKASGYTFTNYGMHWVRQAPGQGLEWMGWINTYSGEATYVDDFQGRVTMTRDTSISTAYMELSRLRSDDTAVYYCLRGYTYQSFDEGGDYWGQGTLVTVSS

SEQ ID NO: 13 - protein, 112 aa, Homo sapiens
DVVMTQSPLSLPVTLGQPASISCRSSQSLLDTDGKTYLNWFQQRPGQSPRRLIYLVSKLDSGVPDRFSGSGSGTDFTLKISRVEAEDVGVYYCWQGTHFPYTFGQGTKLEIK

SEQ ID NO: 14 - protein, 112 aa, Homo sapiens
DVVMTQSPLSLPVTLGQPASISCRSSQSLLDSDAKTYLNWFQQRPGQSPRRLIYLVSKLDSGVPDRFSGSGSGTDFTLKISRVEAEDVGVYYCWQGTHFPYTFGQGTKLEIK

SEQ ID NO: 15 - protein, 112 aa, Homo sapiens
DVVMTQSPLSLPVTLGQPASISCRSSQSLLDTDAKTYLNWFQQRPGQSPRRLIYLVSKLDSGVPDRFSGSGSGTDFTLKISRVEAEDVGVYYCWQGTHFPYTFGQGTKLEIK

SEQ ID NO: 16 - protein, 112 aa, Homo sapiens
DVVMTQSPLSLPVTLGQPASISCRSSQSLLDADGKTYLNWFQQRPGQSPRRLIYLVSKLDSGVPDRFSGSGSGTDFTLKISRVEAEDVGVYYCWQGTHFPYTFGQGTKLEIK

SEQ ID NO: 17 - protein, 112 aa, Homo sapiens
DVVMTQSPLSLPVTLGQPASISCRSSQSLLDNDGKTYLNWFQQRPGQSPRRLIYLVSKLDSGVPDRFSGSGSGTDFTLKISRVEAEDVGVYYCWQGTHFPYTFGQGTKLEIK

SEQ ID NO: 18 - protein, 12 aa, Homo sapiens
  SITE 3: note = X = citrulline
SGXGKQGGKARA

SEQ ID NO: 19 - protein, 23 aa, Homo sapiens
  SITE 3: note = X = citrulline
SGXGKGGKGLGKGGAKRHRKVLR

SEQ ID NO: 20 - protein, 12 aa, Homo sapiens
  SITE 3: note = X = citrulline
SGXGKGGKGLGK

SEQ ID NO: 21 - protein, 12 aa, Homo sapiens
  SITE 6: note = X = citrulline
QFPVGXVHRLLR

SEQ ID NO: 22 - protein, 12 aa, Homo sapiens
  SITE 6: note = X = citrulline
VHRLLXKGNYSE

SEQ ID NO: 23 - protein, 329 aa, Homo sapiens
ASTKGPSVFPLAPSSKSTSGGTAALGCLVKDYFPEPVTVSWNSGALTSGVHTFPAVLQSSGLYSLSSVVTVPSSSLGTQTYICNVNHKPSNTKVDKKVEPKSCDKTHTCPPCPAPELLGGPSVFLFPPKPKDTLMISRTPEVTCVVVDVSHEDPEVKFNWYVDGVEVHNAKTKPREEQYNSTYRVVSVLTVLHQDWLNGKEYKCKVSNKALPAPIEKTISKAKGQPREPQVYTLPPSRDELTKNQVSLTCLVKGFYPSDIAVEWESNGQPENNYKTTPPVLDSDGSFFLYSKLTVDKSRWQQGNVFSCSVMHEALHNHYTQKSLSLSPG

SEQ ID NO: 24 - protein, 107 aa, Homo sapiens [sequence omitted]

SEQ ID NO: 25 - protein, 122 aa, Mus musculus
RIQLVQSGPELKKPGEAVKISCKASGYTFTNYGMHWMKQTPGKDFRWMGWINTYSGEATYVDDFKGRFAFSLGTSASTAYLQINNLKNDDTATYFCLRGYTYQSFDEGGDYWGQGTALTVSS

SEQ ID NO: 26 - protein, 122 aa, Homo sapiens
QVQLVQSGAEVKKPGASVKVSCKASGYTFTNYGMHWVRQAPGQGLEWMGWINTYSGEATYAQKFQGRVTMTRDTSISTAYMELSRLRSDDTAVYYCLRGYTYQSFDEGGDYWGQGTLVTVSS

SEQ ID NO: 27 - protein, 122 aa, Homo sapiens
QVQLVQSGAEVKKPGSSVKVSCKASGYTFTNYGMHWVRQAPGQGLEWMGWINTYSGEATYAQKFQGRVTITADESTSTAYMELSSLRSEDTAVYYCLRGYTYQSFDEGGDYWGQGTLVTVSS

SEQ ID NO: 28 - protein, 122 aa, Homo sapiens
QVQLVQSGAEVKKPGSSVKVSCKASGYTFTNYGMHWVRQAPGQGLEWMGWINTYSGEATYVDDFQGRVTITADESTSTAYMELSSLRSEDTAVYYCLRGYTYQSFDEGGDYWGQGTLVTVSS

SEQ ID NO: 29 - protein, 122 aa, Homo sapiens
QVQLVQSGAEVKKPGASVKVSCKASGYTFTNYGMHWVRQAPGQGLEWMGWINTYSGEATYVDDFQGRVTMTRDTSISTAYMELSRLRSDDTAVYYCLRGYTYQSFDEGGDYWGQGTLVTVSS

SEQ ID NO: 30 - protein, 112 aa, Mus musculus
DVVMTQTPLTLSVTTGQPASISCKSSQSLLDSDGKTYLNWLFQRPGQSPKRLIYLVSKLDSGVPDRFTGSGSGTDFTLKISRVEAEDLGIYYCWQGTHFPYTFGGGTNLEIK

SEQ ID NO: 31 - protein, 112 aa, Homo sapiens
DVVMTQSPLSLPVTLGQPASISCRSSQSLVDSDGKTYLNWFQQRPGQSPRRLIYLVSKLDSGVPDRFSGSGSGTDFTLKISRVEAEDVGVYYCWQGTHFPYTFGQGTKLEIK

SEQ ID NO: 32 - protein, 112 aa, Homo sapiens
DVVMTQSPLSLPVTLGQPASISCRSSQSLLDSDGKTYLNWFQQRPGQSPRRLIYLVSKLDSGVPDRFSGSGSGTDFTLKISRVEAEDVGVYYCWQGTHFPYTFGQGTKLEIK

SEQ ID NO: 33 - protein, 112 aa, Homo sapiens
DVVMTQSPLSLPVTLGQPASISCRSSQSLVASDGKTYLNWFQQRPGQSPRRLIYLVSKLDSGVPDRFSGSGSGTDFTLKISRVEAEDVGVYYCWQGTHFPYTFGQGTKLEIK

SEQ ID NO: 34 - protein, 112 aa, Homo sapiens
DVVMTQSPLSLPVTLGQPASISCRSSQSLVESDGKTYLNWFQQRPGQSPRRLIYLVSKLDSGVPDRFSGSGSGTDFTLKISRVEAEDVGVYYCWQGTHFPYTFGQGTKLEIK

SEQ ID NO: 35 - protein, 112 aa, Homo sapiens
DVVMTQSPLSLPVTLGQPASISCRSSQSLVSSDGKTYLNWFQQRPGQSPRRLIYLVSKLDSGVPDRFSGSGSGTDFTLKISRVEAEDVGVYYCWQGTHFPYTFGQGTKLEIK

SEQ ID NO: 36 - protein, 11 aa, synthetic construct
  REGION 1..11: note = CDR1 of msVL22.101 and hVL22.101g
QSLLDSDGKTY

SEQ ID NO: 37 - protein, 11 aa, Homo sapiens
QSLVDSDGKTY

SEQ ID NO: 38 - protein, 11 aa, Homo sapiens
QSLVASDGKTY

SEQ ID NO: 39 - protein, 11 aa, Homo sapiens
QSLVESDGKTY

SEQ ID NO: 40 - protein, 11 aa, Homo sapiens
QSLVSSDGKTY

SEQ ID NO: 41 - protein, 11 aa, Homo sapiens
QSLLESDGKTY

SEQ ID NO: 42 - protein, 11 aa, Homo sapiens
QSLLDSEGKTY

SEQ ID NO: 43 - protein, 11 aa, Homo sapiens
QSLLDSSGKTY

SEQ ID NO: 44 - protein, 11 aa, Homo sapiens
QSLLESEGKTY

SEQ ID NO: 45 - protein, 11 aa, Homo sapiens
QSLLESSGKTY

SEQ ID NO: 46 - protein, 11 aa, Homo sapiens
QSLLESDAKTY

SEQ ID NO: 47 - protein, 11 aa, Homo sapiens
QSLLDTEGKTY

SEQ ID NO: 48 - protein, 11 aa, Homo sapiens
QSLLDTSGKTY

SEQ ID NO: 49 - protein, 11 aa, Homo sapiens
QSLLDSAGKTY

SEQ ID NO: 50 - protein, 11 aa, Homo sapiens
QSLLESAGKTY

SEQ ID NO: 51 - protein, 11 aa, Homo sapiens
QSLLDAEGKTY

SEQ ID NO: 52 - protein, 11 aa, Homo sapiens
QSLLDNEGKTY

SEQ ID NO: 53 - protein, 17 aa, Homo sapiens
  SITE 9: note = X = citrulline
EPTDSLDAXGHRPVDRR

SEQ ID NO: 54 - protein, 15 aa, Homo sapiens
  SITE 4: note = X = citrulline
  SITE 9: note = X = citrulline
  SITE 11: note = X = citrulline
YVTXSSAVXLXSSVP

SEQ ID NO: 55 - protein, 7 aa, synthetic construct
  REGION 1..7: note = Region around CDR2 of msVL22.101 and hVL22.101(LC)y
LVSKLDS

SEQ ID NO: 56 - protein, 330 aa, Homo sapiens [sequence omitted]